European Patent Application EP 4 692 355 A1, published February 11, 2026. Title: A neucleic acid construct coding for a insulin receptor fragment, and use thereof. Applicant: Tokyo Metropolitan Institute of Medical Science. The sequence listing filed with the application follows.

SEQUENCE LISTING (7 sequences)

SEQ ID NO: 1 - DNA, 63 bp, Homo sapiens
  source 1..63: mol_type = genomic DNA
gccatgagcaaagatggtaaaaagaagaaaaagaagtcaaagacaaagtgtgtaattatgtaa

SEQ ID NO: 2 - DNA, 1215 bp, Mus musculus
  source 1..1215: mol_type = genomic DNA
tttctgagaaagaggcagccggatgggccaatgggaccactgtatgcatcttcaaaccctgagtacctcagtgccagtgatgtgtttccatcttctgtgtacgtgccggacgagtgggaggtgcctcgagagaagatcacccttcttcgagagctggggcagggatcctttggtatggtgtatgaaggcaatgccaaggatatcatcaagggtgaggcagagacccgtgttgcggttaagactgtcaatgagtcagccagtcttcgagaacggatcgagttcctcaatgaggcatcagtcatgaagggattcacctgccatcatgtggtccgccttcttggggtggtatccaaaggacagccaacgctggtagtgatggaattgatggctcatggagacctgaaaagtcacctccgttctctgaggccagatgctgagaataacccaggccgccctccccctaccttgcaagaaatgattcagatgacagcagaaattgctgatggcatggcatacttgaacgccaagaagtttgtgcaccgggacctggcagctcgaaactgcatggttgcccatgattttactgtcaaaattggagactttggaatgacaagggacatctacgagacagattactatcggaaagggggcaagggactgcttcctgtgaggtggatgtcacctgagtccctgaaggatggagtctttactgcttcttctgatatgtggtcctttggggtggtcctttgggaaatcactagcctggctgagcaaccttatcaaggcctgtctaatgaacaggtgttgaagtttgtcatggatggaggctatctggatccccctgataactgtccagagagactcactgacctgatgcgcatgtgctggcagttcaaccccaagatgaggccaaccttcctggaaatcgtcaacctgctcaaggatgacctccaccccagctttccagaagtttccttcttctacagcgaggagaacaaggctcctgagagtgaggagctggagatggagtttgaagacatggagaatgtcccgttggatcgttcctctcactgtcagagagaagaggctgggggccgggagggagggtcctcactgagcatcaaacggacctatgatgaacacatcccctatacccacatgaatgggggcaagaagaacggacgtgtccttaccctgccaaggtcaaacccttcc

SEQ ID NO: 3 - DNA, 1284 bp, synthetic construct
  source 1..1284: mol_type = other DNA
tttctgagaaagaggcagccggatgggccaatgggaccactgtatgcatcttcaaaccctgagtacctcagtgccagtgatgtgtttccatcttctgtgtacgtgccggacgagtgggaggtgcctcgagagaagatcacccttcttcgagagctggggcagggatcctttggtatggtgtatgaaggcaatgccaaggatatcatcaagggtgaggcagagacccgtgttgcggttaagactgtcaatgagtcagccagtcttcgagaacggatcgagttcctcaatgaggcatcagtcatgaagggattcacctgccatcatgtggtccgccttcttggggtggtatccaaaggacagccaacgctggtagtgatggaattgatggctcatggagacctgaaaagtcacctccgttctctgaggccagatgctgagaataacccaggccgccctccccctaccttgcaagaaatgattcagatgacagcagaaattgctgatggcatggcatacttgaacgccaagaagtttgtgcaccgggacctggcagctcgaaactgcatggttgcccatgattttactgtcaaaattggagactttggaatgacaagggacatctacgagacagattactatcggaaagggggcaagggactgcttcctgtgaggtggatgtcacctgagtccctgaaggatggagtctttactgcttcttctgatatgtggtcctttggggtggtcctttgggaaatcactagcctggctgagcaaccttatcaaggcctgtctaatgaacaggtgttgaagtttgtcatggatggaggctatctggatccccctgataactgtccagagagactcactgacctgatgcgcatgtgctggcagttcaaccccaagatgaggccaaccttcctggaaatcgtcaacctgctcaaggatgacctccaccccagctttccagaagtttccttcttctacagcgaggagaacaaggctcctgagagtgaggagctggagatggagtttgaagacatggagaatgtcccgttggatcgttcctctcactgtcagagagaagaggctgggggccgggagggagggtcctcactgagcatcaaacggacctatgatgaacacatcccctatacccacatgaatgggggcaagaagaacggacgtgtccttaccctgccaaggtcaaacccttcctctagagccatgagcaaagatggtaaaaagaagaaaaagaagtcaaagacaaagtgtgtaattatgtaa

SEQ ID NO: 4 - protein, 20 aa, Homo sapiens
AMSKDGKKKKKKSKTKCVIM

SEQ ID NO: 5 - protein, 405 aa, Mus musculus
FLRKRQPDGPMGPLYASSNPEYLSASDVFPSSVYVPDEWEVPREKITLLRELGQGSFGMVYEGNAKDIIKGEAETRVAVKTVNESASLRERIEFLNEASVMKGFTCHHVVRLLGVVSKGQPTLVVMELMAHGDLKSHLRSLRPDAENNPGRPPPTLQEMIQMTAEIADGMAYLNAKKFVHRDLAARNCMVAHDFTVKIGDFGMTRDIYETDYYRKGGKGLLPVRWMSPESLKDGVFTASSDMWSFGVVLWEITSLAEQPYQGLSNEQVLKFVMDGGYLDPPDNCPERLTDLMRMCWQFNPKMRPTFLEIVNLLKDDLHPSFPEVSFFYSEENKAPESEELEMEFEDMENVPLDRSSHCQREEAGGREGGSSLSIKRTYDEHIPYTHMNGGKKNGRVLTLPRSNPS

SEQ ID NO: 6 - protein, 427 aa, synthetic construct
FLRKRQPDGPMGPLYASSNPEYLSASDVFPSSVYVPDEWEVPREKITLLRELGQGSFGMVYEGNAKDIIKGEAETRVAVKTVNESASLRERIEFLNEASVMKGFTCHHVVRLLGVVSKGQPTLVVMELMAHGDLKSHLRSLRPDAENNPGRPPPTLQEMIQMTAEIADGMAYLNAKKFVHRDLAARNCMVAHDFTVKIGDFGMTRDIYETDYYRKGGKGLLPVRWMSPESLKDGVFTASSDMWSFGVVLWEITSLAEQPYQGLSNEQVLKFVMDGGYLDPPDNCPERLTDLMRMCWQFNPKMRPTFLEIVNLLKDDLHPSFPEVSFFYSEENKAPESEELEMEFEDMENVPLDRSSHCQREEAGGREGGSSLSIKRTYDEHIPYTHMNGGKKNGRVLTLPRSNPSSRAMSKDGKKKKKKSKTKCVIM

SEQ ID NO: 7 - protein, 405 aa, Homo sapiens
FLRKRQPDGPLGPLYASSNPEYLSASDVFPCSVYVPDEWEVSREKITLLRELGQGSFGMVYEGNARDIIKGEAETRVAVKTVNESASLRERIEFLNEASVMKGFTCHHVVRLLGVVSKGQPTLVVMELMAHGDLKSYLRSLRPEAENNPGRPPPTLQEMIQMAAEIADGMAYLNAKKFVHRDLAARNCMVAHDFTVKIGDFGMTRDIYETDYYRKGGKGLLPVRWMAPESLKDGVFTTSSDMWSFGVVLWEITSLAEQPYQGLSNEQVLKFVMDGGYLDQPDNCPERVTDLMRMCWQFNPKMRPTFLEIVNLLKDDLHPSFPEVSFFHSEENKAPESEELEMEFEDMENVPLDRSSHCQREEAGGRDGGSSLGFKRSYEEHIPYTHMNGGKKNGRILTLPRSNPS